European Patent Application EP 4 279 076 A1, published November 22, 2023. Title: RNA molecule, Chimeric NA molecule, Double-stranded RNA molecule, and Double-stranded Chimeric NA molecule. Applicant: The University of Tokyo. The sequence listing filed with the application follows.

SEQUENCE LISTING (239 sequences)

SEQ ID NO: 1 - RNA, 21 nt, Artificial Sequence
  siRNA forward
gggagcugauggccuaggaaa

SEQ ID NO: 2 - RNA, 21 nt, Artificial Sequence
  (6)...(8) 2'-O-methyl-modified
uccuaggccaucagcucccac

SEQ ID NO: 3 - RNA, 21 nt, Artificial Sequence
  (6) and (8) 2'-O-methyl-modified
uccuaggccaucagcucccac

SEQ ID NO: 4 - DNA, 33 bp, Artificial Sequence
  reporter forward
tggtagttggagctggtggcgtaggcaagagtg

SEQ ID NO: 5 - DNA, 33 bp, Artificial Sequence
  reporter reverse
cactcttgcctacgccaccagctccaactacca

SEQ ID NO: 6 - DNA, 33 bp, Artificial Sequence
  reporter forward
tggtagttggagctgatggcgtaggcaagagtg

SEQ ID NO: 7 - DNA, 33 bp, Artificial Sequence
  reporter reverse
cactcttgcctacgccatcagctccaactacca

SEQ ID NO: 8 - DNA, 21 bp, Artificial Sequence
  siRNA forward
guuggagcugauggcguagtt

SEQ ID NO: 9 - DNA, 21 bp, Artificial Sequence
  siRNA reverse
cuacgccaucagcuccaactt

SEQ ID NO: 10 - RNA, 21 nt, Artificial Sequence
  siRNA forward
uuggagcugauggcguaggca

SEQ ID NO: 11 - RNA, 21 nt, Artificial Sequence
  siRNA reverse
ccuacgccaucagcuccaacu

SEQ ID NO: 12 - RNA, 21 nt, Artificial Sequence
  siRNA forward
uggagcugauggcguaggcaa

SEQ ID NO: 13 - RNA, 21 nt, Artificial Sequence
  siRNA reverse
gccuacgccaucagcuccaac

SEQ ID NO: 14 - RNA, 21 nt, Artificial Sequence
  siRNA forward
gggagcugauggcguaggaaa

SEQ ID NO: 15 - RNA, 21 nt, Artificial Sequence
  siRNA reverse
uccuacgccaucagcucccac

SEQ ID NO: 16 - RNA, 21 nt, Artificial Sequence
  siRNA forward
gggagcugauggcguaggaaa

SEQ ID NO: 17 - RNA, 21 nt, Artificial Sequence
  siRNA reverse (2)...(5) 2'-O-methyl modified
uccuacgccaucagcucccac

SEQ ID NO: 18 - RNA, 21 nt, Artificial Sequence
  siRNA forward
gggagcugauggcguaggaaa

SEQ ID NO: 19 - RNA, 21 nt, Artificial Sequence
  siRNA reverse (6)...(8) 2'-O-methyl modified
uccuacgccaucagcucccac

SEQ ID NO: 20 - RNA, 21 nt, Artificial Sequence
  siRNA forward
gggagcugauggcguacgaaa

SEQ ID NO: 21 - RNA, 21 nt, Artificial Sequence
  siRNA reverse
ucguacgccaucagcucccac

SEQ ID NO: 22 - RNA, 21 nt, Artificial Sequence
  siRNA forward
gggagcugauggcguuggaaa

SEQ ID NO: 23 - RNA, 21 nt, Artificial Sequence
  siRNA reverse
uccaacgccaucagcucccac

SEQ ID NO: 24 - RNA, 21 nt, Artificial Sequence
  siRNA forward
gggagcugauggcgaaggaaa

SEQ ID NO: 25 - RNA, 21 nt, Artificial Sequence
  siRNA reverse
uccuucgccaucagcucccac

SEQ ID NO: 26 - RNA, 21 nt, Artificial Sequence
  siRNA forward
gggagcugauggccuaggaaa

SEQ ID NO: 27 - RNA, 21 nt, Artificial Sequence
  siRNA reverse
uccuaggccaucagcucccac

SEQ ID NO: 28 - RNA, 21 nt, Artificial Sequence
  siRNA forward
gggagcugaugggguaggaaa

SEQ ID NO: 29 - RNA, 21 nt, Artificial Sequence
  siRNA reverse
uccuaccccaucagcucccac

SEQ ID NO: 30 - RNA, 21 nt, Artificial Sequence
  siRNA forward
gggagcugauggcguacgaaa

SEQ ID NO: 31 - RNA, 21 nt, Artificial Sequence
  siRNA reverse (6)...(8) 2'-O-methyl modified
ucguacgccaucagcucccac

SEQ ID NO: 32 - RNA, 21 nt, Artificial Sequence
  siRNA forward
gggagcugauggcguuggaaa

SEQ ID NO: 33 - RNA, 21 nt, Artificial Sequence
  siRNA reverse (6)...(8) 2'-O-methly modified
uccaacgccaucagcucccac

SEQ ID NO: 34 - RNA, 21 nt, Artificial Sequence
  siRNA
gggagcugauggcgaaggaaa

SEQ ID NO: 35 - RNA, 21 nt, Artificial Sequence
  siRNA reverse (6)...(8) 2'-O-methyl modified
uccuucgccaucagcucccac

SEQ ID NO: 36 - RNA, 21 nt, Artificial Sequence
  siRNA forward
gggagcugauggccuaggaaa

SEQ ID NO: 37 - RNA, 21 nt, Artificial Sequence
  siRNA reverse (6)...(8) 2'-O-methyl modified
uccuaggccaucagcucccac

SEQ ID NO: 38 - RNA, 21 nt, Artificial Sequence
  siRNA forward
gggagcugaugggguaggaaa

SEQ ID NO: 39 - RNA, 21 nt, Artificial Sequence
  siRNA reverse (6)...(8) 2'-O-methyl modified
uccuaccccaucagcucccac

SEQ ID NO: 40 - DNA, 33 bp, Artificial Sequence
  reporter forward
tggtagttggagctgttggcgtaggcaagagtg

SEQ ID NO: 41 - DNA, 33 bp, Artificial Sequence
  reporter reverse
cactcttgcctacgccaacagctccaactacca

SEQ ID NO: 42 - DNA, 33 bp, Artificial Sequence
  reporter forward
tggtagttggagctgctggcgtaggcaagagtg

SEQ ID NO: 43 - DNA, 33 bp, Artificial Sequence
  reporter reverse
cactcttgcctacgccagcagctccaactacca

SEQ ID NO: 44 - RNA, 21 nt, Artificial Sequence
  siRNA forward
gggagcuguuggcguaggaaa

SEQ ID NO: 45 - RNA, 21 nt, Artificial Sequence
  siRNA reverse
uccuacgccaacagcucccac

SEQ ID NO: 46 - RNA, 21 nt, Artificial Sequence
  siRNA forward
gggagcuguuggcgaaggaaa

SEQ ID NO: 47 - RNA, 21 nt, Artificial Sequence
  siRNA reverse (6)...(8) 2'-O-methyl modified
uccuucgccaacagcucccac

SEQ ID NO: 48 - RNA, 21 nt, Artificial Sequence
  siRNA forward
gggagcuguuggccuaggaaa

SEQ ID NO: 49 - RNA, 21 nt, Artificial Sequence
  siRNA reverse (6)...(8) 2'-O-methyl modified
uccuaggccaacagcucccac

SEQ ID NO: 50 - RNA, 21 nt, Artificial Sequence
  siRNA forward
gggagcugcuggcguaggaaa

SEQ ID NO: 51 - RNA, 21 nt, Artificial Sequence
  siRNA reverse
uccuacgccagcagcucccac

SEQ ID NO: 52 - RNA, 21 nt, Artificial Sequence
  siRNA forward
gggagcugcuggcgaaggaaa

SEQ ID NO: 53 - RNA, 21 nt, Artificial Sequence
  siRNA reverse (6)...(8) 2'-O-methyl modified
uccuucgccagcagcucccac

SEQ ID NO: 54 - RNA, 21 nt, Artificial Sequence
  siRNA forward
gggagcugcuggccuaggaaa

SEQ ID NO: 55 - RNA, 21 nt, Artificial Sequence
  siRNA reverse (6)...(8) 2'-O-methyl modified
uccuaggccagcagcucccac

SEQ ID NO: 56 - DNA, 40 bp, Artificial Sequence
  reporter forward
actggtggtggttggagcaggtggtgttgggaaaagcgca

SEQ ID NO: 57 - DNA, 40 bp, Artificial Sequence
  reporter reverse
tgcgcttttcccaacaccaccagctccaaccaccaccagt

SEQ ID NO: 58 - DNA, 40 bp, Artificial Sequence
  reporter forward
actggtggtggttggagcagatggtgttgggaaaagcgca

SEQ ID NO: 59 - DNA, 40 bp, Artificial Sequence
  reporter reverse
tgcgcttttcccaacaccatcagctccaaccaccaccagt

SEQ ID NO: 60 - RNA, 21 nt, Artificial Sequence
  siRNA forward
uggagcaggugguguugggaa

SEQ ID NO: 61 - RNA, 21 nt, Artificial Sequence
  siRNA reverse
cccaacaccaccugcuccaac

SEQ ID NO: 62 - RNA, 21 nt, Artificial Sequence
  siRNA forward
uggagcagaugguguugggaa

SEQ ID NO: 63 - RNA, 21 nt, Artificial Sequence
  siRNA reverse
cccaacaccaucugcuccaac

SEQ ID NO: 64 - RNA, 21 nt, Artificial Sequence
  siRNA forward
cggagcagauggugauggaaa

SEQ ID NO: 65 - RNA, 21 nt, Artificial Sequence
  siRNA reverse (6)...(8) 2'-O-methyl modified
uccaucaccaucugcuccgac

SEQ ID NO: 66 - DNA, 38 bp, Artificial Sequence
  reporter forward
catactggatacagctggacaagaagagtacagtgcca

SEQ ID NO: 67 - DNA, 38 bp, Artificial Sequence
  reporter reverse
tggcactgtactcttcttgtccagctgtatccagtatg

SEQ ID NO: 68 - DNA, 38 bp, Artificial Sequence
  reporter forward
catactggatacagctggacgagaagagtacagtgcca

SEQ ID NO: 69 - DNA, 38 bp, Artificial Sequence
  reporter reverse
tggcactgtactcttctcgtccagctgtatccagtatg

SEQ ID NO: 70 - RNA, 21 nt, Artificial Sequence
  siRNA forward
agcuggacaagaagaguacag

SEQ ID NO: 71 - RNA, 21 nt, Artificial Sequence
  siRNA reverse
guacucuucuuguccagcugu

SEQ ID NO: 72 - RNA, 21 nt, Artificial Sequence
  siRNA forward
agcuggacgagaagaguacag

SEQ ID NO: 73 - RNA, 21 nt, Artificial Sequence
  siRNA reverse
guacucuucucguccagcugu

SEQ ID NO: 74 - RNA, 21 nt, Artificial Sequence
  siRNA forward
ggcuggacgagaaguguaaag

SEQ ID NO: 75 - RNA, 21 nt, Artificial Sequence
  siRNA reverse (6)...(8) 2'-O-methyl modified
uuacacuucucguccagccgu

SEQ ID NO: 76 - DNA, 47 bp, Artificial Sequence
  reporter sense strand
tcgaggttaagagatccccacagtacttcaacgctagaagaacacag

SEQ ID NO: 77 - DNA, 47 bp, Artificial Sequence
  reporter antisense strand
aattctgtgttcttctagcgttgaagtactgtggggatctcttaacc

SEQ ID NO: 78 - DNA, 47 bp, Artificial Sequence
  reporter sense strand
tcgaggttaagagatccccacagtaattcaacgctagaagaacacag

SEQ ID NO: 79 - DNA, 47 bp, Artificial Sequence
  reporter antisense strand
aattctgtgttcttctagcgttgaattactgtggggatctcttaacc

SEQ ID NO: 80 - DNA, 47 bp, Artificial Sequence
  reporter sense strand
tcgagccggagcctttggaagtctgcgcccttgtgccctgcctccag

SEQ ID NO: 81 - DNA, 47 bp, Artificial Sequence
  reporter antisense strand
aattctggaggcagggcacaagggcgcagacttccaaaggctccggc

SEQ ID NO: 82 - DNA, 47 bp, Artificial Sequence
  reporter sense strand
tcgagccggagcctttggaagtctgtgcccttgtgccctgcctccag

SEQ ID NO: 83 - DNA, 47 bp, Artificial Sequence
  reporter antisense strand
aattctggaggcagggcacaagggcacagacttccaaaggctccggc

SEQ ID NO: 84 - DNA, 47 bp, Artificial Sequence
  reporter sense strand
tcgagcccacgcctgctccctcatctactgtgtgcacttcatcctgg

SEQ ID NO: 85 - DNA, 47 bp, Artificial Sequence
  reporter antisense strand
aattccaggatgaagtgcacacagtagatgagggagcaggcgtgggc

SEQ ID NO: 86 - DNA, 47 bp, Artificial Sequence
  reporter sense strand
tcgagcccacgcctgctccctcatccactgtgtgcacttcatcctgg

SEQ ID NO: 87 - DNA, 47 bp, Artificial Sequence
  reporter antisense strand
aattccaggatgaagtgcacacagtggatgagggagcaggcgtgggc

SEQ ID NO: 88 - DNA, 47 bp, Artificial Sequence
  reporter sense strand
tcgagagcagcagcagcagcagcagggggacctatcaggacagagtg

SEQ ID NO: 89 - DNA, 47 bp, Artificial Sequence
  reporter antisense strand
aattcactctgtcctgataggtccccctgctgctgctgctgctgctc

SEQ ID NO: 90 - DNA, 47 bp, Artificial Sequence
  reporter sense strand
tcgagagcagcagcagcagcagcagcgggacctatcaggacagagtg

SEQ ID NO: 91 - DNA, 47 bp, Artificial Sequence
  reporter antisense strand
aattcactctgtcctgataggtcccgctgctgctgctgctgctgctc

SEQ ID NO: 92 - DNA, 47 bp, Artificial Sequence
  reporter sense strand
tcgagtgctggagaccatccactggcgtgggcagatccgtcatttcg

SEQ ID NO: 93 - DNA, 47 bp, Artificial Sequence
  reporter antisense strand
aattcgaaatgacggatctgcccacgccagtggatggtctccagcac

SEQ ID NO: 94 - DNA, 47 bp, Artificial Sequence
  reporter sense strand
tcgagtgctggagaccatccactggtgtgggcagatccgtcatttcg

SEQ ID NO: 95 - DNA, 47 bp, Artificial Sequence
  reporter antisense strand
aattcgaaatgacggatctgcccacagcagtggatggtctccagcac

SEQ ID NO: 96 - DNA, 47 bp, Artificial Sequence
  reporter sense strand
tcgaggaatccattctggtgccactaccacagctccttctctgagtg

SEQ ID NO: 97 - DNA, 47 bp, Artificial Sequence
  reporter antisense strand
aattcactcagagaaggagctgtggtagtggcaccagaatggattcc

SEQ ID NO: 98 - DNA, 47 bp, Artificial Sequence
  reporter sense strand
tcgaggaatccattctggtgccactgccacagctccttctctgagtg

SEQ ID NO: 99 - DNA, 47 bp, Artificial Sequence
  reporter antisense strand
aattcactcagagaaggagctgtggcagtggcaccagaatggattcc

SEQ ID NO: 100 - DNA, 47 bp, Artificial Sequence
  reporter sense strand
tcgagaccccgccgcctgctgctgacgggcacaccgctgcagaacag

SEQ ID NO: 101 - DNA, 47 bp, Artificial Sequence
  reporter antisense strand
aattctgttctgcagcggtgtgcccgtcagcagcaggcggcggggtc

SEQ ID NO: 102 - DNA, 47 bp, Artificial Sequence
  reporter sense strand
tcgagaccccgccgcctgctgctgatgggcacaccgctgcagaacag

SEQ ID NO: 103 - DNA, 47 bp, Artificial Sequence
  reporter antisense strand
aattctgttctgcagcggtgtgcccatcagcagcaggcggcggggtc

SEQ ID NO: 104 - DNA, 47 bp, Artificial Sequence
  reporter sense strand
tcgagtggccccaatcggcctggtgctcatcgtgggaggctacttcg

SEQ ID NO: 105 - DNA, 47 bp, Artificial Sequence
  reporter antisense strand
aattcgaagtagcctcccacgatgagcaccaggccgattggggccac

SEQ ID NO: 106 - DNA, 47 bp, Artificial Sequence
  reporter sense strand
tcgagtggccccaatcggcctggtgttcatcgtgggaggctacttcg

SEQ ID NO: 107 - DNA, 47 bp, Artificial Sequence
  reporter antisense strand
aattcgaagtagcctcccacgatgaacaccaggccgattggggccac

SEQ ID NO: 108 - DNA, 47 bp, Artificial Sequence
  reporter sense strand
tcgagcaaggccttgcctggcttccgcaacttacacgtggacgaccg

SEQ ID NO: 109 - DNA, 47 bp, Artificial Sequence
  reporter antisense strand
aattcggtcgtccacgtgtaagttgcggaagccaggcaaggccttgc

SEQ ID NO: 110 - DNA, 47 bp, Artificial Sequence
  reporter sense strand
tcgagcaaggccttgcctggcttcctcaacttacacgtggacgaccg

SEQ ID NO: 111 - DNA, 47 bp, Artificial Sequence
  reporter antisense strand
aattcggtcgtccacgtgtaagttgaggaagccaggcaaggccttgc

SEQ ID NO: 112 - DNA, 47 bp, Artificial Sequence
  reporter sense strand
tcgaggaatcaatcgcatcttccacgagcggttcccatttgagctgg

SEQ ID NO: 113 - DNA, 47 bp, Artificial Sequence
  reporter antisense strand
aattccagctcaaatgggaaccgctcgtggaagatgcgattgattcc

SEQ ID NO: 114 - DNA, 47 bp, Artificial Sequence
  reporter sense strand
tcgaggaatcaatcgcatcttccacaagcggttcccatttgagctgg

SEQ ID NO: 115 - DNA, 47 bp, Artificial Sequence
  reporter antisense strand
aattccagctcaaatgggaaccgcttgtggaagatgcgattgattcc

SEQ ID NO: 116 - DNA, 47 bp, Artificial Sequence
  reporter sense strand
tcgagtcaagaccctcaacaacaagtttgcctccttcatcgacaagg

SEQ ID NO: 117 - DNA, 47 bp, Artificial Sequence
  reporter antisense strand
aattccttgtcgatgaaggaggcaaacttgttgttgagggtcttgac

SEQ ID NO: 118 - DNA, 47 bp, Artificial Sequence
  reporter sense strand
tcgagtcaagaccctcaacaacaaggttgcctccttcatcgacaagg

SEQ ID NO: 119 - DNA, 47 bp, Artificial Sequence
  reporter antisense strand
aattccttgtcgatgaaggaggcaaccttgttgttgagggtcttgac

SEQ ID NO: 120 - DNA, 47 bp, Artificial Sequence
  reporter sense strand
tcgagtctccgaagcccacacgtgtatccctgagaacaacggaggcg

SEQ ID NO: 121 - DNA, 47 bp, Artificial Sequence
  reporter antisense strand
aattcgcctccgttgttctcagggatacacgtgtgggcttcggagac

SEQ ID NO: 122 - DNA, 47 bp, Artificial Sequence
  reporter sense strand
tcgagtctccgaagcccacacgtgtgtccctgagaacaacggaggcg

SEQ ID NO: 123 - DNA, 47 bp, Artificial Sequence
  reporter antisense strand
aattcgcctccgttgttctcagggacacacgtgtgggcttcggagac

SEQ ID NO: 124 - DNA, 47 bp, Artificial Sequence
  reporter sense strand
tcgagcttaccgcagcttcagcaactccctgagccagtcaccgtgtg

SEQ ID NO: 125 - DNA, 47 bp, Artificial Sequence
  reporter antisense strand
aattcacacggtgactggctcagggagttgctgaagctgcggtaagc

SEQ ID NO: 126 - DNA, 47 bp, Artificial Sequence
  reporter sense strand
tcgagcttaccgcagcttcagcaaccccctgagccagtcaccgtgtg

SEQ ID NO: 127 - DNA, 47 bp, Artificial Sequence
  reporter antisense strand
aattcacacggtgactggctcagggggttgctgaagctgcggtaagc

SEQ ID NO: 128 - DNA, 47 bp, Artificial Sequence
  reporter sense strand
tcgagggataatatcaaacacgtcccgggaggcggcagtgtgcaaag

SEQ ID NO: 129 - DNA, 47 bp, Artificial Sequence
  reporter antisense strand
aattctttgcacactgccgcctcccgggacgtgtttgatattatccc

SEQ ID NO: 130 - DNA, 47 bp, Artificial Sequence
  reporter sense strand
tcgagggataatatcaaacacgtcctgggaggcggcagtgtgcaaag

SEQ ID NO: 131 - DNA, 47 bp, Artificial Sequence
  reporter antisense strand
aattctttgcacactgccgcctcccaggacgtgtttgatattatccc

SEQ ID NO: 132 - DNA, 47 bp, Artificial Sequence
  reporter sense strand
tcgagtgagttggaagacccaggggaaatgtctcctcccattgattg

SEQ ID NO: 133 - DNA, 47 bp, Artificial Sequence
  reporter antisense strand
aattcaatcaatgggaggagacatttcccctgggtcttccaactcac

SEQ ID NO: 134 - DNA, 47 bp, Artificial Sequence
  reporter sense strand
tcgagtgagttggaagacccagggggaatgtctcctcccattgattg

SEQ ID NO: 135 - DNA, 47 bp, Artificial Sequence
  reporter antisense strand
aattcaatcaatgggaggagacattccccctgggtcttccaactcac

SEQ ID NO: 136 - DNA, 47 bp, Artificial Sequence
  reporter sense strand
tcgagggcggcggcagcagcagcgggggctgcgggcggtcggggctg

SEQ ID NO: 137 - DNA, 47 bp, Artificial Sequence
  reporter antisense strand
aattcagccccgaccgcccgcagcccccgctgctgctgccgccgccc

SEQ ID NO: 138 - DNA, 47 bp, Artificial Sequence
  reporter sense strand
tcgagggcggcggcagcagcagcggcggctgcgggcggtcggggctg

SEQ ID NO: 139 - DNA, 47 bp, Artificial Sequence
  reporter antisense strand
aattcagccccgaccgcccgcagccgccgctgctgctgccgccgccc

SEQ ID NO: 140 - DNA, 47 bp, Artificial Sequence
  reporter sense strand
tcgaggacgggtgtggtacgcagccccttcgagtacccacagtactg

SEQ ID NO: 141 - DNA, 47 bp, Artificial Sequence
  reporter antisense strand
aattcagtactgtgggtactcgaaggggctgcgtaccacacccgtcc

SEQ ID NO: 142 - DNA, 47 bp, Artificial Sequence
  reporter sense strand
tcgaggacgggtgtggtacgcagccacttcgagtacccacagtactg

SEQ ID NO: 143 - DNA, 47 bp, Artificial Sequence
  reporter antisense strand
aattcagtactgtgggtactcgaagtggctgcgtaccacacccgtcc

SEQ ID NO: 144 - DNA, 47 bp, Artificial Sequence
  reporter sense strand
tcgagcggagacgagccaggtggcctcggcctaagacctgcctaggg

SEQ ID NO: 145 - DNA, 47 bp, Artificial Sequence
  reporter antisense strand
aattccctaggcaggtcttaggccgaggccacctggctcgtctccgc

SEQ ID NO: 146 - DNA, 47 bp, Artificial Sequence
  reporter sense strand
tcgagtgagaacattcagagttctccgagcattgaagacgatttcag

SEQ ID NO: 147 - DNA, 47 bp, Artificial Sequence
  reporter antisense strand
aattctgaaatcgtcttcaatgctcggagaactctgaatgttctcac

SEQ ID NO: 148 - DNA, 47 bp, Artificial Sequence
  reporter sense strand
tcgagtgagaacattcagagttctctgagcattgaagacgatttcag

SEQ ID NO: 149 - DNA, 47 bp, Artificial Sequence
  reporter antisense strand
aattctgaaatcgtcttcaatgctcagagaactctgaatgttctcac

SEQ ID NO: 150 - DNA, 47 bp, Artificial Sequence
  reporter sense strand
tcgagcttgaattccaagagcacacggtcttcagtgaagctgcaggg

SEQ ID NO: 151 - DNA, 47 bp, Artificial Sequence
  reporter antisense strand
aattccctgcagcttcactgaagaccgtgtgctcttggaattcaagc

SEQ ID NO: 152 - DNA, 47 bp, Artificial Sequence
  reporter sense strand
tcgagcttgaattccaagagcacacagtcttcagtgaagctgcaggg

SEQ ID NO: 153 - DNA, 47 bp, Artificial Sequence
  reporter antisense strand
aattccctgcagcttcactgaagactgtgtgctcttggaattcaagc

SEQ ID NO: 154 - DNA, 47 bp, Artificial Sequence
  reporter sense strand
tcgagaccgccgaagcctcagcccacgacccggaccccgcctcagtg

SEQ ID NO: 155 - DNA, 47 bp, Artificial Sequence
  reporter antisense strand
aattcactgaggcggggtccgggtcgtgggctgaggcttcggcggtc

SEQ ID NO: 156 - DNA, 47 bp, Artificial Sequence
  reporter sense strand
tcgagaccgccgaagcctcagcccaggacccggaccccgcctcagtg

SEQ ID NO: 157 - DNA, 47 bp, Artificial Sequence
  reporter antisense strand
aattcactgaggcggggtccgggtcctgggctgaggcttcggcggtc

SEQ ID NO: 158 - DNA, 47 bp, Artificial Sequence
  reporter sense strand
tcgagtgttccgggccctgggcctgcggcacctggtggtggtggacg

SEQ ID NO: 159 - DNA, 47 bp, Artificial Sequence
  reporter antisense strand
aattcgtccaccaccaccaggtgccgcaggcccagggcccggaacac

SEQ ID NO: 160 - DNA, 47 bp, Artificial Sequence
  reporter sense strand
tcgagtgttccgggccctgggcctgtggcacctggtggtggtggacg

SEQ ID NO: 161 - DNA, 47 bp, Artificial Sequence
  reporter antisense strand
aattcgtccaccaccaccaggtgccacaggcccagggcccggaacac

SEQ ID NO: 162 - DNA, 47 bp, Artificial Sequence
  reporter sense strand
tcgagtcccctccatcatgaatgtgctgctggtgtgtctcatcttcg

SEQ ID NO: 163 - DNA, 47 bp, Artificial Sequence
  reporter antisense strand
aattcgaagatgagacacaccagcagcacattcatgatggaggggac

SEQ ID NO: 164 - DNA, 47 bp, Artificial Sequence
  reporter sense strand
tcgagtcccctccatcatgaatgtggtgctggtgtgtctcatcttcg

SEQ ID NO: 165 - DNA, 47 bp, Artificial Sequence
  reporter antisense strand
aattcgaagatgagacacaccagcaccacattcatgatggaggggac

SEQ ID NO: 166 - DNA, 47 bp, Artificial Sequence
  reporter sense strand
tcgagacatcattggtgcctccagcgactgcagcacctgctttgtgg

SEQ ID NO: 167 - DNA, 47 bp, Artificial Sequence
  reporter antisense strand
aattccacaaagcaggtgctgcagtcgctggaggcaccaatgatgtc

SEQ ID NO: 168 - DNA, 47 bp, Artificial Sequence
  reporter sense strand
tcgagacatcattggtgcctccagctactgcagcacctgctttgtgg

SEQ ID NO: 169 - DNA, 47 bp, Artificial Sequence
  reporter antisense strand
aattccacaaagcaggtgctgcagtagctggaggcaccaatgatgtc

SEQ ID NO: 170 - DNA, 47 bp, Artificial Sequence; identical to SEQ ID NO: 116
  reporter sense strand

SEQ ID NO: 171 - DNA, 47 bp, Artificial Sequence; identical to SEQ ID NO: 117
  reporter antisense strand

SEQ ID NO: 172 - DNA, 47 bp, Artificial Sequence; identical to SEQ ID NO: 118
  reporter sense strand

SEQ ID NO: 173 - DNA, 47 bp, Artificial Sequence; identical to SEQ ID NO: 119
  reporter antisense strand

SEQ ID NO: 174 - RNA, 21 nt, Artificial Sequence
  siRNA
ccacaguacuucaacgcuaga

SEQ ID NO: 175 - RNA, 21 nt, Artificial Sequence
  siRNA
uagcguugaaguacugugggg

SEQ ID NO: 176 - RNA, 21 nt, Artificial Sequence
  siRNA
gaagucugcgcccuugugccc

SEQ ID NO: 177 - RNA, 21 nt, Artificial Sequence
  siRNA
gcacaagggcgcagacuucca

SEQ ID NO: 178 - RNA, 21 nt, Artificial Sequence
  siRNA
cccucaucuacugugugcacu

SEQ ID NO: 179 - RNA, 21 nt, Artificial Sequence
  siRNA
ugcacacaguagaugagggag

SEQ ID NO: 180 - RNA, 21 nt, Artificial Sequence
  siRNA
agcagcagggggaccuaucag

SEQ ID NO: 181 - RNA, 21 nt, Artificial Sequence
  siRNA
agcagcagggggaccuaucag

SEQ ID NO: 182 - RNA, 21 nt, Artificial Sequence
  siRNA
uccacuggcgugggcagaucc

SEQ ID NO: 183 - RNA, 21 nt, Artificial Sequence
  siRNA
aucugcccacgccaguggaug

SEQ ID NO: 184 - RNA, 21 nt, Artificial Sequence
  siRNA
gugccacuaccacagcuccuu

SEQ ID NO: 185 - RNA, 21 nt, Artificial Sequence
  siRNA
ggagcugugguaguggcacca

SEQ ID NO: 186 - RNA, 21 nt, Artificial Sequence
  siRNA
gcugcugacgggcacaccgcu

SEQ ID NO: 187 - RNA, 21 nt, Artificial Sequence
  siRNA
cggugugcccgucagcagcag

SEQ ID NO: 188 - RNA, 21 nt, Artificial Sequence
  siRNA
gccuggugcucaucgugggag

SEQ ID NO: 189 - RNA, 21 nt, Artificial Sequence
  siRNA
cccacgaugagcaccaggccg

SEQ ID NO: 190 - RNA, 21 nt, Artificial Sequence
  siRNA
gcacaguaauucaucgcuaga

SEQ ID NO: 191 - RNA, 21 nt, Artificial Sequence
  siRNA
uagcgaugaauuacugugcgg

SEQ ID NO: 192 - RNA, 21 nt, Artificial Sequence
  siRNA
gaagucugugcccaugugacc

SEQ ID NO: 193 - RNA, 21 nt, Artificial Sequence
  siRNA
ucacaugggcacagacuucca

SEQ ID NO: 194 - RNA, 21 nt, Artificial Sequence
  siRNA
gccucauccacugagugcacu

SEQ ID NO: 195 - RNA, 21 nt, Artificial Sequence
  siRNA
ugcacucaguggaugaggcag

SEQ ID NO: 196 - RNA, 21 nt, Artificial Sequence
  siRNA
ggcagcagcgggagcuauaag

SEQ ID NO: 197 - RNA, 21 nt, Artificial Sequence
  siRNA
uauagcucccgcugcugccgc

SEQ ID NO: 198 - RNA, 21 nt, Artificial Sequence
  siRNA
gccacugguguggccagaacc

SEQ ID NO: 199 - RNA, 21 nt, Artificial Sequence
  siRNA
uucuggccacaccaguggcug

SEQ ID NO: 200 - RNA, 21 nt, Artificial Sequence
  siRNA
gugccacugccacugcucauu

SEQ ID NO: 201 - RNA, 21 nt, Artificial Sequence
  siRNA
ugagcaguggcaguggcacca

SEQ ID NO: 202 - RNA, 21 nt, Artificial Sequence
  siRNA
gcugcugaugggcucaccacu

SEQ ID NO: 203 - RNA, 21 nt, Artificial Sequence
  siRNA
uggugagcccaucagcagcag

SEQ ID NO: 204 - RNA, 21 nt, Artificial Sequence
  siRNA
gccugguguucaugguggaag

SEQ ID NO: 205 - RNA, 21 nt, Artificial Sequence
  siRNA
gccaccaugaacaccaggccg

SEQ ID NO: 206 - RNA, 21 nt, Artificial Sequence
  siRNA
gggcuuccucaacauacaagu

SEQ ID NO: 207 - RNA, 21 nt, Artificial Sequence
  siRNA
uuguauguugaggaagcccgg

SEQ ID NO: 208 - RNA, 21 nt, Artificial Sequence
  siRNA
gcuuccacaagcgcuuccaau

SEQ ID NO: 209 - RNA, 21 nt, Artificial Sequence
  siRNA
uggaagcgcuuguggaagcug

SEQ ID NO: 210 - RNA, 21 nt, Artificial Sequence
  siRNA
ggagcagccggccgagcuacg

SEQ ID NO: 211 - RNA, 21 nt, Artificial Sequence
  siRNA
uagcucggccggcugcuccuc

SEQ ID NO: 212 - RNA, 21 nt, Artificial Sequence
  siRNA
gcacgugugucccagagaaca

SEQ ID NO: 213 - RNA, 21 nt, Artificial Sequence
  siRNA
uucucugggacacacgugcgg

SEQ ID NO: 214 - RNA, 21 nt, Artificial Sequence
  siRNA
gcagcaacccccucagccagu

SEQ ID NO: 215 - RNA, 21 nt, Artificial Sequence
  siRNA
uggcugaggggguugcugcag

SEQ ID NO: 216 - RNA, 21 nt, Artificial Sequence
  siRNA
gcacguccugggacgcggaag

SEQ ID NO: 217 - RNA, 21 nt, Artificial Sequence
  siRNA
uccgcgucccaggacgugcuu

SEQ ID NO: 218 - RNA, 21 nt, Artificial Sequence
  siRNA
gccagggggaaugacuccacc

SEQ ID NO: 219 - RNA, 21 nt, Artificial Sequence
  siRNA
uggagucauucccccuggcuc

SEQ ID NO: 220 - RNA, 21 nt, Artificial Sequence
  siRNA
ggcagcggcggcuccgggagg

SEQ ID NO: 221 - RNA, 21 nt, Artificial Sequence
  siRNA
ucccggagccgccgcugccgc

SEQ ID NO: 222 - RNA, 21 nt, Artificial Sequence
  siRNA
gcgcagccacuuccaguaacc

SEQ ID NO: 223 - RNA, 21 nt, Artificial Sequence
  siRNA
uuacuggaaguggcugcgcac

SEQ ID NO: 224 - RNA, 21 nt, Artificial Sequence
  siRNA
ggguggccucggcguaagacc

SEQ ID NO: 225 - RNA, 21 nt, Artificial Sequence
  siRNA
ucuuacgccgaggccacccgg

SEQ ID NO: 226 - RNA, 21 nt, Artificial Sequence
  siRNA
gaguucucugagcuuugaaga

SEQ ID NO: 227 - RNA, 21 nt, Artificial Sequence
  siRNA
uucaaagcucagagaacucug

SEQ ID NO: 228 - RNA, 21 nt, Artificial Sequence
  siRNA
gagcacacagucuacaguaaa

SEQ ID NO: 229 - RNA, 21 nt, Artificial Sequence
  siRNA
uacuguagacugugugcucuu

SEQ ID NO: 230 - RNA, 21 nt, Artificial Sequence
  siRNA
gcagcccaggaccgggacacc

SEQ ID NO: 231 - RNA, 21 nt, Artificial Sequence
  siRNA
ugucccgguccugggcugcgg

SEQ ID NO: 232 - RNA, 21 nt, Artificial Sequence
  siRNA
ggacccggacgccguggacca

SEQ ID NO: 233 - RNA, 21 nt, Artificial Sequence
  siRNA
uccagcugccacaggccccgg

SEQ ID NO: 234 - RNA, 21 nt, Artificial Sequence
  siRNA
ggaauguggugcucguguauc

SEQ ID NO: 235 - RNA, 21 nt, Artificial Sequence
  siRNA
uacacgagcaccacauuccug

SEQ ID NO: 236 - RNA, 21 nt, Artificial Sequence
  siRNA
gcuccagcuacuggagcaacu

SEQ ID NO: 237 - RNA, 21 nt, Artificial Sequence
  siRNA
uugcuccaguagcuggagcca

SEQ ID NO: 238 - RNA, 21 nt, Artificial Sequence
  siRNA
gcaacaagguugcguccuaca

SEQ ID NO: 239 - RNA, 21 nt, Artificial Sequence
  siRNA
uaggacgcaaccuuguugcug